European Patent Application EP 4 692 126 A1, published February 11, 2026. Title: ANTI-5T4 ANTIBODY AND USE THEREOF. Applicant: SOUND BIOPHARMACEUTICALS CO. LTD. Application EP 24784229.7, filed April 1, 2024. The sequence listing filed with the application follows.

SEQUENCE LISTING (19 sequences)

SEQ ID NO: 1 - protein, 6 aa, synthetic construct
QDISNY

SEQ ID NO: 2 - skipped

SEQ ID NO: 3 - protein, 9 aa, synthetic construct
QQGDTVPLT

SEQ ID NO: 4 - protein, 8 aa, synthetic construct
GFTFRNYA

SEQ ID NO: 5 - protein, 8 aa, synthetic construct
ISTGGSYT

SEQ ID NO: 6 - protein, 13 aa, synthetic construct
AFYYYGSSYSMDY

SEQ ID NO: 7 - protein, 107 aa, synthetic construct
DIQMTQTTSSLSASLGDRVTISCRASQDISNYLNWYQQKPDGTVKLLIYHTSILHSGVPSRFSGSGSGTDYSLTISNLEQEDIATYFCQQGDTVPLTFGAGTKLELK

SEQ ID NO: 8 - protein, 120 aa, synthetic construct
EVQLVESGGGLVKPGGSLKLSCAASGFTFRNYAMSWVRQSPDKRLEWVAEISTGGSYTYYPDTVTGRFTISRDNAKNTLYLEMSSLRSEDTAMYYCAFYYYGSSYSMDYWGQGTSVTVSS

SEQ ID NO: 9 - protein, 107 aa, synthetic construct
DIQMTQSPSSLSASVGDRVTISCRASQDISNYLNWYQQKPGKAPKLLIYHTSILHSGVPSRFSGSGSGTDYSLTISSLQPEDIATYFCQQGDTVPLTFGGGTKVEIK

SEQ ID NO: 10 - protein, 107 aa, synthetic construct
DIQMTQSPSSLSASVGDRVTISCRASQDISNYLNWYQQKPGKVPKLLIYHTSILHSGVPSRFSGSGSGTDYSLTISSLQPEDVATYFCQQGDTVPLTFGGGTKVEIK

SEQ ID NO: 11 - protein, 107 aa, synthetic construct
DIQMTQTTSSLSASVGDRVTISCRASQDISNYLNWFQQKPGKAPKSLIYHTSILHSGVPSKFSGSGSGTDYSLTISSLQPEDFATYFCQQGDTVPLTFGGGTKVEIK

SEQ ID NO: 12 - protein, 107 aa, synthetic construct
DIQMTQSPSSLSASVGDRVTISCRASQDISNYLNWYQQKPGKAPKLLIYHTSILHSGVPSRFSGSGSGTDYSLTISSLQPEDFATYFCQQGDTVPLTFGGGTKVEIK

SEQ ID NO: 13 - protein, 120 aa, synthetic construct
EVQLVESGGGLVQPGGSLRLSCAASGFTFRNYAMSWVRQAPGKGLEWVAEISTGGSYTYYPDTVTGRFTISRDNAKNSLYLQMNSLRAEDTAVYYCAFYYYGSSYSMDYWGQGTLVTVSS

SEQ ID NO: 14 - protein, 120 aa, synthetic construct
EVQLVESGGGLVQPGGSLRLSCAASGFTFRNYAMSWVRQAPGKGLEWVAEISTGGSYTYYPDTVTGRFTISRDNSKNTLYLQMNSLRAEDTAVYYCAFYYYGSSYSMDYWGQGTLVTVSS

SEQ ID NO: 15 - protein, 120 aa, synthetic construct
EVQLVESGGGLVQPGGSLRLSCAASGFTFRNYAMSWVRQAPGKGLEWVAEISTGGSYTYYPDTVTGRFTISRDNAKNTLYLQMNSLRAEDTAVYYCAFYYYGSSYSMDYWGQGTLVTVSS

SEQ ID NO: 16 - protein, 120 aa, synthetic construct
EVQLVESGGGVVQPGRSLRLSCAASGFTFRNYAMSWVRQAPGKGLEWVAEISTGGSYTYYPDTVTGRFTISRDNSKNTLYLQMSSLRAEDTAVYYCAFYYYGSSYSMDYWGQGTLVTVSS

SEQ ID NO: 17 - protein, 120 aa, synthetic construct
EVQLVESGGGVVQPGRSLRLSCAASGFTFRNYAMSWVRQAPGKGLEWVAEISTGGSYTYYPDTVTGRFTISRDNAKNTLYLQMNSLRAEDTAVYYCAFYYYGSSYSMDYWGQGTLVTVSS

SEQ ID NO: 18 - protein, 107 aa, Homo sapiens [sequence omitted]

SEQ ID NO: 19 - protein, 330 aa, Homo sapiens [sequence omitted]